European Patent Application EP 4 534 672 A1, published April 9, 2025. Title: A monoclonal antibody binding to CB1. Applicant: SHIONOGI & CO., LTD. Application JP. The sequence listing filed with the application follows.

SEQUENCE LISTING (53 sequences)

SEQ ID NO: 1 - protein, 110 aa, synthetic construct
  REGION 1..110: note = VL of mIML1-2
QIVLTQSPAIMSASPGEKVTMTCRASSSVSSSYLHWYQQKSGASPKLWIYSTSNLASGVPARFSGSGSGTSYSLTITSVEAEDVATYYCQQYSGFPLTFGSGTKLEIKRT

SEQ ID NO: 2 - protein, 110 aa, synthetic construct
  REGION 1..110: note = VL of m20C3
DIVLTQSPAIMSASPGEKVTMTCRASSSVSSSYLHWYQQKSGASPKLWIYSTSNLASGVPARFSGSGSGTSYSLTISSVEAEDAATYYCQQYSGFPLTFGQGTKVEIKRA

SEQ ID NO: 3 - protein, 110 aa, synthetic construct
  REGION 1..110: note = VL of m2F8
QIVLTQSPAIMSASLGERITLTCIASSSVSSSYLHWYQQKPGSSPKLWIYSTSNLASGVPTRFSGSGSGTSFSLTISTMEAEDAATYYCHQYHRSPRTFGGGTKLEIKRA

SEQ ID NO: 4 - protein, 110 aa, synthetic construct
  REGION 1..110: note = VL of m4D7, m24C4, m26C7
QIVLTQSPAIMSASLGERITLTCTASSSVSSSYLHWYQQKPGSSPKLWIYSTSNLASGVPTRFSGSGSGTSFSLTISTMEAEDAATYYCHQYHRSPRTFGGGTKLEIKRA

SEQ ID NO: 5 - protein, 12 aa, synthetic construct
  REGION 1..12: note = VL-CDR1 of Humanized antibody
  SITE 1: note = misc_feature - Xaa can be Ile or Lys or Arg
  SITE 8: note = misc_feature - Xaa can be Ser or Thr
  SITE 9: note = misc_feature - Xaa can be Ser or Arg
XASSSVSXXYLH

SEQ ID NO: 6 - skipped

SEQ ID NO: 7 - protein, 117 aa, synthetic construct
  REGION 1..117: note = VH of mIML1-2
QVQLQQSGAELVKPGASVKIACKASGYEFNYYWMNWVKQRPGKGLEWIGQIYPGDGDNKYNGKFKGKATLTADKSSSTVYMQLNSLTSEDSAVYFCARTGSGRFAYWGQGTLVTVSA

SEQ ID NO: 8 - protein, 117 aa, synthetic construct
  REGION 1..117: note = VH m20C3
QVQLQQSGAELVKPGASVKISCKASGYEFNYYWMNWVKQRPGKGLEWIGQIYPGDADNKYNAKFKGKATLTADKSSSTAYMQLSSLTSEDSAVYFCARTGSGRFAYWGQGTLVTVSA

SEQ ID NO: 9 - protein, 117 aa, synthetic construct
  REGION 1..117: note = VH of m2F8
QVQLQQSGAELVKPGASVKISCKASGYEFSYYWMNWVKQRPGKGLEWIGQIYPGDGDTNYNGKFKGKATLAAGKSSSTAYMQLSSLTSEDSAVYFCARSHGNYMIYWGQGTSVTVSS

SEQ ID NO: 10 - protein, 117 aa, synthetic construct
  REGION 1..117: note = VH of m4D7
QVQLQQSGAELVKPGASVKISCKASGYEFSYYWMNWVKQRPGKGLEWIGQIYPGDGDTNYNGKFKGKATVTADKSSSTAYMQLSSLTSEDSAVYFCAKSHGNYMDYWGQGTSVTVSS

SEQ ID NO: 11 - protein, 117 aa, synthetic construct
  REGION 1..117: note = VH of m24C4
QVQLQQSGAELVKPGASVKISCKASGYEFSYYWMNWVKQRPGKGLEWIGQIYPGDGDTNYNGKFKGKATLTADKSSSTAYMQLSSLTSEDSAVYFCARSHGNYMHYWGQGTSVTVSS

SEQ ID NO: 12 - protein, 117 aa, synthetic construct
  REGION 1..117: note = VH of m26C7
QVQLQQSGAELVKPGASVKISCKASGYEFSYYWMNWVKQRPGKGLEWIGQIYPGDGDTNYNGKFKGKATLTADKSSSTAYMQLSSLTSEDSAVYFCARSHGNYMAYWGQGTSVTVSS

SEQ ID NO: 13 - protein, 110 aa, synthetic construct
  REGION 1..110: note = VL of hIML1-2
DIQMTQSPSSLSASVGDRVTITCRASSSVSSSYLHWYQQKPGKAPKLLIYSTSNLASGVPSRFSGSGSGTDFTLTISSLQPEDFATYYCQQYSGFPLTFGQGTKVEIKRT

SEQ ID NO: 14 - protein, 110 aa, synthetic construct
  REGION 1..110: note = VL of hIML1-2-OP1
DIQMTQSPSSLSASVGDRVTITCKASSSVSTRYLHWYQQKPGKAPKLLIYGTSNIASGVPSRFSGSGSGTDFTLTISSLQPEDVATYYCQQYTAFPLTFGQGTKVEIKRT

SEQ ID NO: 15 - protein, 110 aa, synthetic construct
  REGION 1..110: note = VL of h2F8
EIVLTQSPGTLSLSPGERATLSCIASSSVSSSYLHWYQQKPGQAPRLLIHSTSNLASGIPERFSGSGSGPDFTLTISRLKPEDFAVYYCHQYHRSPRTFGQGTKVEIKRT

SEQ ID NO: 16 - protein, 117 aa, synthetic construct
  REGION 1..117: note = VH of hIML1-2
QVQLVQSGAEVKKPGASVKVSCKASGYTFNYYWMNWVRQAPGQGLEWMGQIYPGDADNKYNAKFKGRVTMTRDTSTSTVYMELSSLRSEDTAVYYCARTGSGRFAYWGQGTLVTVSS

SEQ ID NO: 17 - protein, 117 aa, synthetic construct
  REGION 1..117: note = VH of hIML1-2-OP1
QVQLVQSGAEVKKPGASVKVSCKASGYEFNYYWMNWVRQAPGQGLEWMGQIYPGDGDNRYNGKFKGRVTMTRDTSTSTVYMELSSLRSEDTAVYYCARTGSGRFAYWGQGTLVTVSS

SEQ ID NO: 18 - protein, 117 aa, synthetic construct
  REGION 1..117: note = VH of h2F8
QVQLVQSGAEVKKPGASVKVSCKASGYEFSYYWMNWVRQAPGQGLEWMGQIYPGDGDTNYNGKFKGRVTMTRDTSTSTVYMELSSLRSEDTAVYYCARSHGNYMIYWGQGTTVTVSS

SEQ ID NO: 19 - protein, 12 aa, synthetic construct
  REGION 1..12: note = VL-CDR1 of mIML1-2, m20C3, hIML1-2
RASSSVSSSYLH

SEQ ID NO: 20 - protein, 7 aa, synthetic construct
  REGION 1..7: note = VL-CDR2 of mIML1-2, m20C3, m2F8, m4D7, m24C4, m26C7, hIML1-2, h2F8
STSNLAS

SEQ ID NO: 21 - protein, 9 aa, synthetic construct
  REGION 1..9: note = VL-CDR3 of mIML1-2, m20C3, hIML1-2
QQYSGFPLT

SEQ ID NO: 22 - protein, 12 aa, synthetic construct
  REGION 1..12: note = VL-CDR1 of m4D7, m24C4, m26C7
TASSSVSSSYLH

SEQ ID NO: 23 - protein, 9 aa, synthetic construct
  REGION 1..9: note = VL-CDR3 of m2F8, m4D7, m24C4, m26C7, h2F8
HQYHRSPRT

SEQ ID NO: 24 - protein, 5 aa, synthetic construct
  REGION 1..5: note = VH-CDR1 of mIML1-2, m20C3, m2F8, m4D7, m24C4, m26C7, hIML1-2, hIML1-2-OP1, h2F8
YYWMN

SEQ ID NO: 25 - protein, 17 aa, synthetic construct
  REGION 1..17: note = VH-CDR2 of mIML1-2
QIYPGDGDNKYNGKFKG

SEQ ID NO: 26 - protein, 8 aa, synthetic construct
  REGION 1..8: note = VH-CDR3 of mIML1-2, m20C3, hIML1-2, hIML1-2-OP1
TGSGRFAY

SEQ ID NO: 27 - protein, 17 aa, synthetic construct
  REGION 1..17: note = VH-CDR2 of m20C3, hIML1-2
QIYPGDADNKYNAKFKG

SEQ ID NO: 28 - protein, 17 aa, synthetic construct
  REGION 1..17: note = VH-CDR2 of m2F8, m4D7, m24C4, m26C7, h2F8
QIYPGDGDTNYNGKFKG

SEQ ID NO: 29 - protein, 8 aa, synthetic construct
  REGION 1..8: note = VH-CDR3 of m2F8, h2F8
SHGNYMIY

SEQ ID NO: 30 - protein, 8 aa, synthetic construct
  REGION 1..8: note = VH-CDR3 of m4D7
SHGNYMDY

SEQ ID NO: 31 - protein, 8 aa, synthetic construct
  REGION 1..8: note = VH-CDR3 of m24C4
SHGNYMHY

SEQ ID NO: 32 - protein, 8 aa, synthetic construct
  REGION 1..8: note = VH-CDR3 of m26C7
SHGNYMAY

SEQ ID NO: 33 - protein, 12 aa, synthetic construct
  REGION 1..12: note = VL-CDR1 of hIML1-2-OP1
KASSSVSTRYLH

SEQ ID NO: 34 - protein, 7 aa, synthetic construct
  REGION 1..7: note = VL-CDR2 of hIML1-2-OP1
GTSNIAS

SEQ ID NO: 35 - protein, 9 aa, synthetic construct
  REGION 1..9: note = VL-CDR3 of hIML1-2-OP1
QQYTAFPLT

SEQ ID NO: 36 - protein, 17 aa, synthetic construct
  REGION 1..17: note = VH-CDR2 of hIML1-2-OP1
QIYPGDGDNRYNGKFKG

SEQ ID NO: 37 - protein, 327 aa, synthetic construct
  REGION 1..327: note = Heavy chain constant region
ASTKGPSVFPLAPCSRSTSESTAALGCLVKDYFPEPVTVSWNSGALTSGVHTFPAVLQSSGLYSLSSVVTVPSSSLGTKTYTCNVDHKPSNTKVDKRVESKYGPPCPPCPAPEFLGGPSVFLFPPKPKDTLMISRTPEVTCVVVDVSQEDPEVQFNWYVDGVEVHNAKTKPREEQFNSTYRVVSVLTVLHQDWLNGKEYKCKVSNKGLPSSIEKTISKAKGQPREPQVYTLPPSQEEMTKNQVSLTCLVKGFYPSDIAVEWESNGQPENNYKTTPPVLDSDGSFFLYSRLTVDKSRWQEGNVFSCSVMHEALHNHYTQKSLSLSLGK

SEQ ID NO: 38 - protein, 105 aa, synthetic construct [sequence omitted]

SEQ ID NO: 39 - protein, 12 aa, synthetic construct
  REGION 1..12: note = VL-CDR1
  SITE 1: note = misc_feature - Xaa can be Thr or Ile or Arg or Lys
  SITE 8: note = misc_feature - Xaa can be Ser or Thr
  SITE 9: note = misc_feature - Xaa can be Ser or Arg
XASSSVSXXYLH

SEQ ID NO: 40 - protein, 12 aa, synthetic construct
  REGION 1..12: note = VL-CDR1 of m2F8, h2F8
IASSSVSSSYLH

SEQ ID NO: 41 - protein, 9 aa, synthetic construct
  REGION 1..9: note = VL-CDR3
  SITE 1: note = misc_feature - Xaa can be His or Glu
  SITE 4: note = misc_feature - Xaa can be His or Thr or Ser
  SITE 5: note = misc_feature - Xaa can be Arg or Ala or Gly
  SITE 6: note = misc_feature - Xaa can be Ser or Phe
  SITE 8: note = misc_feature - Xaa can be Arg or Leu
XQYXXXPXT

SEQ ID NO: 42 - protein, 17 aa, synthetic construct
  REGION 1..17: note = VH-CDR2
  SITE 7: note = misc_feature - Xaa can be Gly or Ala
  SITE 9: note = misc_feature - Xaa can be Thr or Asp
  SITE 10: note = misc_feature - Xaa can be Asp or Lys or Arg
  SITE 13: note = misc_feature - Xaa can be Gly or Ala
QIYPGDXDXXYNXKFKG

SEQ ID NO: 43 - skipped

SEQ ID NO: 44 - protein, 12 aa, synthetic construct
  REGION 1..12: note = VL-CDR1 of IML1-2
  SITE 1: note = misc_feature - Xaa can be Arg or Lys
  SITE 8: note = misc_feature - Xaa can be Thr or Ser
  SITE 9: note = misc_feature - Xaa can be Arg or Ser
XASSSVSXXYLH

SEQ ID NO: 45 - protein, 7 aa, synthetic construct
  REGION 1..7: note = VL-CDR2
  SITE 1: note = misc_feature - Xaa can be Gly or Ser
  SITE 5: note = misc_feature - Xaa can be Leu or Ile
XTSNXAS

SEQ ID NO: 46 - protein, 9 aa, synthetic construct
  REGION 1..9: note = VL-CDR3 of IML1-2
  SITE 4: note = misc_feature - Xaa can be Thr or Ser
  SITE 5: note = misc_feature - Xaa can be Ala or Gly
QQYXXFPLT

SEQ ID NO: 47 - protein, 17 aa, synthetic construct
  REGION 1..17: note = VH-CDR2 of IML1-2
  SITE 7: note = misc_feature - Xaa can be Gly or Ala
  SITE 10: note = misc_feature - Xaa can be Lys or Arg
  SITE 13: note = misc_feature - Xaa can be Gly or Ala
QIYPGDXDNXYNXKFKG

SEQ ID NO: 48 - protein, 12 aa, synthetic construct
  REGION 1..12: note = VL-CDR1 of mouse antibody
  SITE 1: note = misc_feature - Xaa can be Thr or Ile or Arg
XASSSVSSSYLH

SEQ ID NO: 49 - protein, 9 aa, synthetic construct
  REGION 1..9: note = VL-CDR3 of mouse antibody
  SITE 1: note = misc_feature - Xaa can be His or Glu
  SITE 4: note = misc_feature - Xaa can be His or Ser
  SITE 5: note = misc_feature - Xaa can be Arg or Gly
  SITE 6: note = misc_feature - Xaa can be Ser or Phe
  SITE 8: note = misc_feature - Xaa can be Arg or Leu
XQYXXXPXT

SEQ ID NO: 50 - protein, 17 aa, synthetic construct
  REGION 1..17: note = VH-CDR2 of mouse antibody
  SITE 7: note = misc_feature - Xaa can be Gly or Ala
  SITE 9: note = misc_feature - Xaa can be Thr or Asp
  SITE 10: note = misc_feature - Xaa can be Asp or Lys
  SITE 13: note = misc_feature - Xaa can be Gly or Ala
QIYPGDXDXXYNXKFKG

SEQ ID NO: 51 - protein, 472 aa, Homo sapiens
MKSILDGLADTTFRTITTDLLYVGSNDIQYEDIKGDMASKLGYFPQKFPLTSFRGSPFQEKMTAGDNPQLVPADQVNITEFYNKSLSSFKENEENIQCGENFMDIECFMVLNPSQQLAIAVLSLTLGTFTVLENLLVLCVILHSRSLRCRPSYHFIGSLAVADLLGSVIFVYSFIDFHVFHRKDSRNVFLFKLGGVTASFTASVGSLFLTAIDRYISIHRPLAYKRIVTRPKAVVAFCLMWTIAIVIAVLPLLGWNCEKLQSVCSDIFPHIDETYLMFWIGVTSVLLLFIVYAYMYILWKAHSHAVRMIQRGTQKSIIIHTSEDGKVQVTRPDQARMDIRLAKTLVLILVVLIICWGPLLAIMVYDVFGKMNKLIKTVFAFCSMLCLLNSTVNPIIYALRSKDLRHAFRSMFPSCEGTAQPLDNSMGDSDCLHKHANNAASVHRAAESCIKSTVKIAKVTMSVSTDTSAEAL

SEQ ID NO: 52 - protein, 117 aa, synthetic construct
  REGION 1..117: note = VH of hIML1-2-2
QVQLVQSGAEVKKPGASVKVSCKASGYTFNYYWMNWVRQAPGQGLEWMGQIYPGDGDNKYNGKFKGRVTMTRDTSTSTVYMELSSLRSEDTAVYYCARTGSGRFAYWGQGTLVTVSS

SEQ ID NO: 53 - protein, 8 aa, synthetic construct
  REGION 1..8: note = peptide tag
DYKDDDDK